European Patent Specification EP 3 856 894 B1, published August 2, 2023. Title: METHODS FOR DIFFERETIATING MESENCHYMAL STEM CELLS. Applicant: Bone Therapeutics SA. The sequence listing filed with the application follows.

SEQUENCE LISTING (26 sequences)

SEQ ID NO: 1 - DNA, 20 bp, artificial sequence
  Runx2 forward primer
ggttccagcaggtagctgag

SEQ ID NO: 2 - DNA, 20 bp, artificial sequence
  Runx2 reverse primer
agacaccaaactccacagcc

SEQ ID NO: 3 - DNA, 20 bp, artificial sequence
  SOX9 forward primer
taaaggcaactcgtacccaa

SEQ ID NO: 4 - DNA, 20 bp, artificial sequence
  SOX9 reverse primer
attctccatcatcctccacg

SEQ ID NO: 5 - DNA, 20 bp, artificial sequence
  BMP2 forward primer
ggaacggacattcggtcctt

SEQ ID NO: 6 - DNA, 21 bp, artificial sequence
  BMP2 reverse primer
caccatggtcgacctttagga

SEQ ID NO: 7 - DNA, 24 bp, artificial sequence
  ALPL forward primer
accattcccacgtcttcacatttg

SEQ ID NO: 8 - DNA, 22 bp, artificial sequence
  ALPL reverse primer
agacattctctcgttcaccgcc

SEQ ID NO: 9 - DNA, 21 bp, artificial sequence
  MMP13 forward primer
tggaattaaggagcatggcga

SEQ ID NO: 10 - DNA, 20 bp, artificial sequence
  MMP13 reverse primer
aactcatgcgcagcaacaag

SEQ ID NO: 11 - DNA, 23 bp, artificial sequence
  CHI3L1 forward primer
tgggtctcaaagattttccaaga

SEQ ID NO: 12 - DNA, 20 bp, artificial sequence
  CHI3L1 reverse primer
gctgtttgtctctccgtcca

SEQ ID NO: 13 - DNA, 22 bp, artificial sequence
  DCN forward primer
aaaatgcccaaaactcttcagg

SEQ ID NO: 14 - DNA, 21 bp, artificial sequence
  DCN reverse primer
gccccattttcaattcctgag

SEQ ID NO: 15 - DNA, 18 bp, artificial sequence
  OCN forward primer
aaggtgcagcctttgtgt

SEQ ID NO: 16 - DNA, 20 bp, artificial sequence
  OCN reverse primer
gctcccagccattgatacag

SEQ ID NO: 17 - DNA, 19 bp, artificial sequence
  SPON1 forward primer
cctgcggaactgccaagta

SEQ ID NO: 18 - DNA, 19 bp, artificial sequence
  SPON1 reverse primer
cacgggtgagcccaattct

SEQ ID NO: 19 - DNA, 20 bp, artificial sequence
  POSTN forward primer
tttgggcaccaaaaagaaat

SEQ ID NO: 20 - DNA, 22 bp, artificial sequence
  POSTN reverse primer
ttctcatataaccagggcaaca

SEQ ID NO: 21 - DNA, 20 bp, artificial sequence
  RPL13 forward primer
cataggaagctgggagcaag

SEQ ID NO: 22 - DNA, 20 bp, artificial sequence
  RPL13 reverse primer
gccctccaatcagtcttctg

SEQ ID NO: 23 - DNA, 20 bp, artificial sequence
  TBP forward primer
aacaacagcctgccacctta

SEQ ID NO: 24 - DNA, 20 bp, artificial sequence
  TBP reverse primer
gccataaggcatcattggac

SEQ ID NO: 25 - DNA, 19 bp, artificial sequence
  HPRT forward primer
ccctggcgtcgtgattagt

SEQ ID NO: 26 - DNA, 21 bp, artificial sequence
  HPRT reverse primer
gtgatggcctcccatctcctt